European Patent Specification EP 3 504 341 B1, published May 14, 2025. Title: Methods of identifying microsatellite instability. Applicant: The University of Newcastle upon Tyne. The sequence listing filed with the application follows.

SEQUENCE LISTING (337 sequences)

SEQ ID NO: 1 - DNA, 19 bp, Artificial Sequence
  Primer
tgcatgcaagacaggagcc

SEQ ID NO: 2 - DNA, 24 bp, Artificial Sequence
  Primer
ggagaaacaaacttaccttgggaa

SEQ ID NO: 3 - DNA, 21 bp, Artificial Sequence
  Primer
ctttagaactggatccagtgg

SEQ ID NO: 4 - DNA, 20 bp, Artificial Sequence
  Primer
aaaaagtggagtggaggagg

SEQ ID NO: 5 - DNA, 21 bp, Artificial Sequence
  Primer
aacccagtttctttccttctg

SEQ ID NO: 6 - DNA, 20 bp, Artificial Sequence
  Primer
gcctcaacctaggacccttc

SEQ ID NO: 7 - DNA, 20 bp, Artificial Sequence
  Primer
tcaccactggggactttttc

SEQ ID NO: 8 - DNA, 21 bp, Artificial Sequence
  Primer
tgagcacaccaagtcattctg

SEQ ID NO: 9 - DNA, 20 bp, Artificial Sequence
  Primer
tagaggcagcaggctctcag

SEQ ID NO: 10 - DNA, 20 bp, Artificial Sequence
  Primer
accccacaaaccatgaaatc

SEQ ID NO: 11 - DNA, 18 bp, Artificial Sequence
  Primer
cacagcccattcctggac

SEQ ID NO: 12 - DNA, 21 bp, Artificial Sequence
  Primer
gccattgcttacatctcatgg

SEQ ID NO: 13 - DNA, 20 bp, Artificial Sequence
  Primer
aggactctggcacctacgtc

SEQ ID NO: 14 - DNA, 20 bp, Artificial Sequence
  Primer
tcgcaaggaaactacagcag

SEQ ID NO: 15 - DNA, 20 bp, Artificial Sequence
  Primer
tctgggaaaaagcccataac

SEQ ID NO: 16 - DNA, 20 bp, Artificial Sequence
  Primer
acaacaccctctcacccaac

SEQ ID NO: 17 - DNA, 25 bp, Artificial Sequence
  Primer
tgactatgacaggagcttaaaactg

SEQ ID NO: 18 - DNA, 23 bp, Artificial Sequence
  Primer
cccacaccacattgtatgtagac

SEQ ID NO: 19 - DNA, 20 bp, Artificial Sequence
  Primer
ggcacaccaggagaaagagg

SEQ ID NO: 20 - DNA, 19 bp, Artificial Sequence
  Primer
gccccgacctaccatacag

SEQ ID NO: 21 - DNA, 20 bp, Artificial Sequence
  Primer
cgtttttgtggaagcatacg

SEQ ID NO: 22 - DNA, 22 bp, Artificial Sequence
  Primer
ccaaatggcaaataaaagaagg

SEQ ID NO: 23 - DNA, 20 bp, Artificial Sequence
  Primer
catgatatgcccatgtaggg

SEQ ID NO: 24 - DNA, 20 bp, Artificial Sequence
  Primer
attggtgaaggaaccagcag

SEQ ID NO: 25 - DNA, 20 bp, Artificial Sequence
  Primer
cagctgaaaccgaagtgaag

SEQ ID NO: 26 - DNA, 22 bp, Artificial Sequence
  Primer
ttgatgatccttttgacaccac

SEQ ID NO: 27 - DNA, 21 bp, Artificial Sequence
  Primer
ccctttacaccacatcaatgc

SEQ ID NO: 28 - DNA, 18 bp, Artificial Sequence
  Primer
gcagggcccatcatacag

SEQ ID NO: 29 - DNA, 24 bp, Artificial Sequence
  Primer
ttcccaactgtaagaacaagagag

SEQ ID NO: 30 - DNA, 24 bp, Artificial Sequence
  Primer
cacttcagagtgatgttgtcttca

SEQ ID NO: 31 - DNA, 22 bp, Artificial Sequence
  Primer
tcttccttatgacaacccacac

SEQ ID NO: 32 - DNA, 20 bp, Artificial Sequence
  Primer
gagcaccttccgactcactc

SEQ ID NO: 33 - DNA, 23 bp, Artificial Sequence
  Primer
tgccaatatttcaatttttctcc

SEQ ID NO: 34 - DNA, 20 bp, Artificial Sequence
  Primer
agactatgccttgcccagag

SEQ ID NO: 35 - DNA, 25 bp, Artificial Sequence
  Primer
tccaataggaaactgagagctattc

SEQ ID NO: 36 - DNA, 21 bp, Artificial Sequence
  Primer
tggagcagagcaatagagagg

SEQ ID NO: 37 - DNA, 18 bp, Artificial Sequence
  Primer
ctgcagagccacccattc

SEQ ID NO: 38 - DNA, 20 bp, Artificial Sequence
  Primer
agatgaaccaagccagaagc

SEQ ID NO: 39 - DNA, 20 bp, Artificial Sequence
  Primer
tggaggcctcactatgttcc

SEQ ID NO: 40 - DNA, 18 bp, Artificial Sequence
  Primer
ctggtgcacggactatgc

SEQ ID NO: 41 - DNA, 18 bp, Artificial Sequence
  Primer
gtggggacagacccagtg

SEQ ID NO: 42 - DNA, 20 bp, Artificial Sequence
  Primer
gggcaagaggcctaacagtg

SEQ ID NO: 43 - DNA, 20 bp, Artificial Sequence
  Primer
cacagactggttttgcaacg

SEQ ID NO: 44 - DNA, 20 bp, Artificial Sequence
  Primer
cttgtgctccttgctcacag

SEQ ID NO: 45 - DNA, 20 bp, Artificial Sequence
  Primer
ctccagcgagaaagaattgg

SEQ ID NO: 46 - DNA, 19 bp, Artificial Sequence
  Primer
attgatccctcaccggaac

SEQ ID NO: 47 - DNA, 23 bp, Artificial Sequence
  Primer
tttgttatatcccattaggtgcc

SEQ ID NO: 48 - DNA, 20 bp, Artificial Sequence
  Primer
atcacgaggttgagatcgag

SEQ ID NO: 49 - DNA, 22 bp, Artificial Sequence
  Primer
tcaaggccaggcaattaatcag

SEQ ID NO: 50 - DNA, 21 bp, Artificial Sequence
  Primer
acttgctgaatgtccaaggtg

SEQ ID NO: 51 - DNA, 22 bp, Artificial Sequence
  Primer
gtgctacatgagatagctggga

SEQ ID NO: 52 - DNA, 23 bp, Artificial Sequence
  Primer
ctcttctggccagttctatgtgt

SEQ ID NO: 53 - DNA, 22 bp, Artificial Sequence
  Primer
tggagtaagaccctttaggcag

SEQ ID NO: 54 - DNA, 21 bp, Artificial Sequence
  Primer
agactctggaagcaaatggca

SEQ ID NO: 55 - DNA, 20 bp, Artificial Sequence
  Primer
ccttttggccagaatatgcc

SEQ ID NO: 56 - DNA, 20 bp, Artificial Sequence
  Primer
ggcatgaggaagtgaaggga

SEQ ID NO: 57 - DNA, 21 bp, Artificial Sequence
  Primer
aggtgtcaagcaaggactcag

SEQ ID NO: 58 - DNA, 20 bp, Artificial Sequence
  Primer
aggcgttttcacgttggagg

SEQ ID NO: 59 - DNA, 22 bp, Artificial Sequence
  Primer
agaggcagaatgtggaaaagtc

SEQ ID NO: 60 - DNA, 20 bp, Artificial Sequence
  Primer
gcattctcccacagcacaat

SEQ ID NO: 61 - DNA, 22 bp, Artificial Sequence
  Primer
ggagggacatgtgtttccaaat

SEQ ID NO: 62 - DNA, 21 bp, Artificial Sequence
  Primer
cacaatgagccaagtctcaca

SEQ ID NO: 63 - DNA, 23 bp, Artificial Sequence
  Primer
agcaacctcttaaatccagtact

SEQ ID NO: 64 - DNA, 20 bp, Artificial Sequence
  Primer
tgggctttcttgactttgga

SEQ ID NO: 65 - DNA, 23 bp, Artificial Sequence
  Primer
tttctcaggacaaagagcaaggt

SEQ ID NO: 66 - DNA, 20 bp, Artificial Sequence
  Primer
ctgggttccatcttgtgggg

SEQ ID NO: 67 - DNA, 20 bp, Artificial Sequence
  Primer
atcagctgactccttaccct

SEQ ID NO: 68 - DNA, 20 bp, Artificial Sequence
  Primer
tggggtgagagatggacatg

SEQ ID NO: 69 - DNA, 25 bp, Artificial Sequence
  Primer
ctcatggttaatacaattaggcaca

SEQ ID NO: 70 - DNA, 20 bp, Artificial Sequence
  Primer
acatggtgtgctacctttca

SEQ ID NO: 71 - DNA, 21 bp, Artificial Sequence
  Primer
ttcttcagggcccattattgt

SEQ ID NO: 72 - DNA, 21 bp, Artificial Sequence
  Primer
tgaggaatgtgcagttgacac

SEQ ID NO: 73 - DNA, 20 bp, Artificial Sequence
  Primer
agcttggccatatttgtgca

SEQ ID NO: 74 - DNA, 23 bp, Artificial Sequence
  Primer
acttgatagggttaaatgtccgt

SEQ ID NO: 75 - DNA, 21 bp, Artificial Sequence
  Primer
tgccttcgagtttaaatgcct

SEQ ID NO: 76 - DNA, 20 bp, Artificial Sequence
  Primer
gcctcgttattttgtgtgcc

SEQ ID NO: 77 - DNA, 21 bp, Artificial Sequence
  Primer
gccacactgactttgaacctt

SEQ ID NO: 78 - DNA, 22 bp, Artificial Sequence
  Primer
acagcttcttcctcactctact

SEQ ID NO: 79 - DNA, 23 bp, Artificial Sequence
  Primer
tccctagaaagagaacgacaaca

SEQ ID NO: 80 - DNA, 23 bp, Artificial Sequence
  Primer
aaatgcccaccaagattgtaaaa

SEQ ID NO: 81 - DNA, 20 bp, Artificial Sequence
  Primer
ggggagaagacggttgaact

SEQ ID NO: 82 - DNA, 20 bp, Artificial Sequence
  Primer
actggttcactggccttttg

SEQ ID NO: 83 - DNA, 23 bp, Artificial Sequence
  Primer
aggtaaagtcagacacaatccca

SEQ ID NO: 84 - DNA, 21 bp, Artificial Sequence
  Primer
accctcatgtttcccacctca

SEQ ID NO: 85 - DNA, 23 bp, Artificial Sequence
  Primer
gcaatcacatttgcattggtttt

SEQ ID NO: 86 - DNA, 23 bp, Artificial Sequence
  Primer
tgactatgagctccacaaacgta

SEQ ID NO: 87 - DNA, 23 bp, Artificial Sequence
  Primer
ttctccattggaagtatttggga

SEQ ID NO: 88 - DNA, 20 bp, Artificial Sequence
  Primer
tgtgtattcagggtccaggg

SEQ ID NO: 89 - DNA, 21 bp, Artificial Sequence
  Primer
tcataaccaagagcaccacct

SEQ ID NO: 90 - DNA, 21 bp, Artificial Sequence
  Primer
tgtgatagggaaacacacgga

SEQ ID NO: 91 - DNA, 22 bp, Artificial Sequence
  Primer
cagcataaatccaatggctatg

SEQ ID NO: 92 - DNA, 20 bp, Artificial Sequence
  Primer
tcagattgcaaaggggtaca

SEQ ID NO: 93 - DNA, 20 bp, Artificial Sequence
  Primer
aaacatttcgactggtgcaa

SEQ ID NO: 94 - DNA, 20 bp, Artificial Sequence
  Primer
ttcttctttcccccaaatga

SEQ ID NO: 95 - DNA, 20 bp, Artificial Sequence
  Primer
tgggattagggaagggagag

SEQ ID NO: 96 - DNA, 19 bp, Artificial Sequence
  Primer
ggccctccccaactaaaat

SEQ ID NO: 97 - DNA, 20 bp, Artificial Sequence
  Primer
ccttcctttgatccgcaagc

SEQ ID NO: 98 - DNA, 20 bp, Artificial Sequence
  Primer
ctgccacctaggaactggag

SEQ ID NO: 99 - DNA, 20 bp, Artificial Sequence
  Primer
tttttgttgcccatttcctc

SEQ ID NO: 100 - DNA, 21 bp, Artificial Sequence
  Primer
agggtactgaccctagctcca

SEQ ID NO: 101 - DNA, 23 bp, Artificial Sequence
  Primer
ctcagacaaagacatacgaagcc

SEQ ID NO: 102 - DNA, 25 bp, Artificial Sequence
  Primer
ttggttctacagtaattgtgcttct

SEQ ID NO: 103 - DNA, 20 bp, Artificial Sequence
  Primer
ccctcccaaatgtcaagtgt

SEQ ID NO: 104 - DNA, 20 bp, Artificial Sequence
  Primer
cccacccacactcttttgtt

SEQ ID NO: 105 - DNA, 25 bp, Artificial Sequence
  Primer
tcaatgctattggcctataaagagt

SEQ ID NO: 106 - DNA, 20 bp, Artificial Sequence
  Primer
atgcatttccttctggccta

SEQ ID NO: 107 - DNA, 20 bp, Artificial Sequence
  Primer
tcaccatcatcaccatgctt

SEQ ID NO: 108 - DNA, 20 bp, Artificial Sequence
  Primer
tctggcaaactcttcactgg

SEQ ID NO: 109 - DNA, 20 bp, Artificial Sequence
  Primer
agtggagaaaacggttgtgg

SEQ ID NO: 110 - DNA, 20 bp, Artificial Sequence
  Primer
gaaggcagacaagggattca

SEQ ID NO: 111 - DNA, 20 bp, Artificial Sequence
  Primer
gtgaccgcacaaagtcacac

SEQ ID NO: 112 - DNA, 21 bp, Artificial Sequence
  Primer
tccaacaatcacagtccatga

SEQ ID NO: 113 - DNA, 20 bp, Artificial Sequence
  Primer
tcaagactcagccatttcca

SEQ ID NO: 114 - DNA, 21 bp, Artificial Sequence
  Primer
ggaagctgagagcaggttttt

SEQ ID NO: 115 - DNA, 20 bp, Artificial Sequence
  Primer
tcgtcaggctctgcaactac

SEQ ID NO: 116 - DNA, 20 bp, Artificial Sequence
  Primer
cgatgggattgaatttggat

SEQ ID NO: 117 - DNA, 20 bp, Artificial Sequence
  Primer
aggacctcgagcttctcttt

SEQ ID NO: 118 - DNA, 20 bp, Artificial Sequence
  Primer
ttcttttgcttccgtgtgtg

SEQ ID NO: 119 - DNA, 21 bp, Artificial Sequence
  Primer
tgcaaccagaggttttaatcg

SEQ ID NO: 120 - DNA, 20 bp, Artificial Sequence
  Primer
ctcaattcagcaacaggtca

SEQ ID NO: 121 - DNA, 20 bp, Artificial Sequence
  Primer
caaccacagtttgccagcta

SEQ ID NO: 122 - DNA, 22 bp, Artificial Sequence
  Primer
tccttgctatcatttggagaga

SEQ ID NO: 123 - DNA, 21 bp, Artificial Sequence
  Primer
ccagtttcacatttcgcttgt

SEQ ID NO: 124 - DNA, 22 bp, Artificial Sequence
  Primer
tggcaacaaaacagtaacagga

SEQ ID NO: 125 - DNA, 20 bp, Artificial Sequence
  Primer
agtgaatgggctttggactg

SEQ ID NO: 126 - DNA, 20 bp, Artificial Sequence
  Primer
aactggagtgggtgaacctg

SEQ ID NO: 127 - DNA, 20 bp, Artificial Sequence
  Primer
caccagcttttctcccttca

SEQ ID NO: 128 - DNA, 21 bp, Artificial Sequence
  Primer
tggcactcaataccaaactgg

SEQ ID NO: 129 - DNA, 21 bp, Artificial Sequence
  Primer
ggtttctgtgctgaatcttgg

SEQ ID NO: 130 - DNA, 20 bp, Artificial Sequence
  Primer
aaccccagttttctgcctct

SEQ ID NO: 131 - DNA, 20 bp, Artificial Sequence
  Primer
ccatggtaccactgtggagt

SEQ ID NO: 132 - DNA, 20 bp, Artificial Sequence
  Primer
tagagggggcttgaatgttg

SEQ ID NO: 133 - DNA, 20 bp, Artificial Sequence
  Primer
gggctcgacttgatttacga

SEQ ID NO: 134 - DNA, 20 bp, Artificial Sequence
  Primer
gggaagcaatctcatggcta

SEQ ID NO: 135 - DNA, 20 bp, Artificial Sequence
  Primer
acgcatggaaaaagaggttc

SEQ ID NO: 136 - DNA, 20 bp, Artificial Sequence
  Primer
caaggctggtatgggtcaat

SEQ ID NO: 137 - DNA, 20 bp, Artificial Sequence
  Primer
tgtggaatccctcctgaaat

SEQ ID NO: 138 - DNA, 20 bp, Artificial Sequence
  Primer
ccgctggtggacttttactc

SEQ ID NO: 139 - DNA, 20 bp, Artificial Sequence
  Primer
gccaaaatgcctaactccaa

SEQ ID NO: 140 - DNA, 20 bp, Artificial Sequence
  Primer
ggactcggatggaagacaaa

SEQ ID NO: 141 - DNA, 20 bp, Artificial Sequence
  Primer
agggtatgatttgggggtgt

SEQ ID NO: 142 - DNA, 20 bp, Artificial Sequence
  Primer
gtggaccaaaggagcagaag

SEQ ID NO: 143 - DNA, 20 bp, Artificial Sequence
  Primer
tgagggtggatgcttcattt

SEQ ID NO: 144 - DNA, 24 bp, Artificial Sequence
  Primer
caggatattcctcagttcagttcc

SEQ ID NO: 145 - DNA, 21 bp, Artificial Sequence
  Primer
tcaaatgcagactcaacatga

SEQ ID NO: 146 - DNA, 20 bp, Artificial Sequence
  Primer
agcagaggagccatcaattc

SEQ ID NO: 147 - DNA, 20 bp, Artificial Sequence
  Primer
caggcacacacactttcgtt

SEQ ID NO: 148 - DNA, 21 bp, Artificial Sequence
  Primer
ttctcatgcagtcaaccattg

SEQ ID NO: 149 - DNA, 20 bp, Artificial Sequence
  Primer
agacgtccaaaggtcgctaa

SEQ ID NO: 150 - DNA, 20 bp, Artificial Sequence
  Primer
ccctcactgcctgtaaacct

SEQ ID NO: 151 - DNA, 20 bp, Artificial Sequence
  Primer
atcacaaaaacaggggccta

SEQ ID NO: 152 - DNA, 20 bp, Artificial Sequence
  Primer
ccttgtctggctcaatcacc

SEQ ID NO: 153 - DNA, 20 bp, Artificial Sequence
  Primer
ctgctccacattcccattct

SEQ ID NO: 154 - DNA, 20 bp, Artificial Sequence
  Primer
tggcaggaaacatctgttca

SEQ ID NO: 155 - DNA, 21 bp, Artificial Sequence
  Primer
tggctgagtaaaatggtgaca

SEQ ID NO: 156 - DNA, 20 bp, Artificial Sequence
  Primer
gcttgggggaatttcttgat

SEQ ID NO: 157 - DNA, 20 bp, Artificial Sequence
  Primer
cagaaggtcaggaccacaca

SEQ ID NO: 158 - DNA, 20 bp, Artificial Sequence
  Primer
atttggtgggttccagtgag

SEQ ID NO: 159 - DNA, 21 bp, Artificial Sequence
  Primer
cctcctagcattccatagcac

SEQ ID NO: 160 - DNA, 21 bp, Artificial Sequence
  Primer
tgcaacctcgtaagctcattt

SEQ ID NO: 161 - DNA, 20 bp, Artificial Sequence
  Primer
gccacatttgctggtattca

SEQ ID NO: 162 - DNA, 20 bp, Artificial Sequence
  Primer
tttttcctctgggaaaccat

SEQ ID NO: 163 - DNA, 23 bp, Artificial Sequence
  Primer
tggttcagacatacacgtacagg

SEQ ID NO: 164 - DNA, 20 bp, Artificial Sequence
  Primer
ataacaggcacaagggtgga

SEQ ID NO: 165 - DNA, 21 bp, Artificial Sequence
  Primer
cctggcaaatgatgctttaga

SEQ ID NO: 166 - DNA, 20 bp, Artificial Sequence
  Primer
cctccctcctaggctcaagt

SEQ ID NO: 167 - DNA, 20 bp, Artificial Sequence
  Primer
cgaggcgggtatttacttga

SEQ ID NO: 168 - DNA, 20 bp, Artificial Sequence
  Primer
ggagttggggcaaaaatcac

SEQ ID NO: 169 - DNA, 18 bp, Artificial Sequence
  Primer
caaacccccgagacacac

SEQ ID NO: 170 - DNA, 21 bp, Artificial Sequence
  Primer
aacgtggctctttatcccatt

SEQ ID NO: 171 - DNA, 20 bp, Artificial Sequence
  Primer
gatggagggccctttaattt

SEQ ID NO: 172 - DNA, 21 bp, Artificial Sequence
  Primer
cgatgaagtggttgatgtgag

SEQ ID NO: 173 - DNA, 20 bp, Artificial Sequence
  Primer
gacaactccgaagggcaata

SEQ ID NO: 174 - DNA, 20 bp, Artificial Sequence
  Primer
agtttgggttgcaagacgtt

SEQ ID NO: 175 - DNA, 20 bp, Artificial Sequence
  Primer
gcaacattgaaatgctggaa

SEQ ID NO: 176 - DNA, 20 bp, Artificial Sequence
  Primer
taacatttgggagggggaat

SEQ ID NO: 177 - DNA, 20 bp, Artificial Sequence
  Primer
gctgaatagcgggatcaaaa

SEQ ID NO: 178 - DNA, 24 bp, Artificial Sequence
  Primer
ggaattaggtaccagatctccttt

SEQ ID NO: 179 - DNA, 20 bp, Artificial Sequence
  Primer
gattatcagcccagggaggt

SEQ ID NO: 180 - DNA, 20 bp, Artificial Sequence
  Primer
atggcagcactgggaaatta

SEQ ID NO: 181 - DNA, 20 bp, Artificial Sequence
  Primer
tatggctgcagcattaccag

SEQ ID NO: 182 - DNA, 20 bp, Artificial Sequence
  Primer
gccagagtccacagactcaa

SEQ ID NO: 183 - DNA, 20 bp, Artificial Sequence
  Primer
gagcaaggcatttgaatctg

SEQ ID NO: 184 - DNA, 20 bp, Artificial Sequence
  Primer
atatgaggcgctctctctcg

SEQ ID NO: 185 - DNA, 20 bp, Artificial Sequence
  Primer
tgcctttggttgtacctttg

SEQ ID NO: 186 - DNA, 20 bp, Artificial Sequence
  Primer
tcaagtgagccttgtggaaa

SEQ ID NO: 187 - DNA, 20 bp, Artificial Sequence
  Primer
ccttccccgttctttctctt

SEQ ID NO: 188 - DNA, 20 bp, Artificial Sequence
  Primer
aaggtaggtgaccggctgat

SEQ ID NO: 189 - DNA, 20 bp, Artificial Sequence
  Primer
gcatctcaaactgtgcctgt

SEQ ID NO: 190 - DNA, 20 bp, Artificial Sequence
  Primer
cacgggtctaactgtcctca

SEQ ID NO: 191 - DNA, 20 bp, Artificial Sequence
  Primer
ccactccagcaagtctccag

SEQ ID NO: 192 - DNA, 20 bp, Artificial Sequence
  Primer
caagggcctgctgtatgtca

SEQ ID NO: 193 - DNA, 20 bp, Artificial Sequence
  Primer
agcccatgttttccacagaa

SEQ ID NO: 194 - DNA, 20 bp, Artificial Sequence
  Primer
taccaggtgccctaaacagg

SEQ ID NO: 195 - DNA, 21 bp, Artificial Sequence
  Primer
ttctagacacagacgcacacg

SEQ ID NO: 196 - DNA, 21 bp, Artificial Sequence
  Primer
gggactgccactagtagctca

SEQ ID NO: 197 - DNA, 20 bp, Artificial Sequence
  Primer
tgggggcagtttctattctg

SEQ ID NO: 198 - DNA, 20 bp, Artificial Sequence
  Primer
atcagttttcgatggggaga

SEQ ID NO: 199 - DNA, 20 bp, Artificial Sequence
  Primer
ttggatgctggattttgaca

SEQ ID NO: 200 - DNA, 20 bp, Artificial Sequence
  Primer
ctcatatccccctcccagaa

SEQ ID NO: 201 - DNA, 20 bp, Artificial Sequence
  Primer
tattggccaggaatttttgc

SEQ ID NO: 202 - DNA, 20 bp, Artificial Sequence
  Primer
ggagctcacgctaatgacct

SEQ ID NO: 203 - DNA, 20 bp, Artificial Sequence
  Primer
ccccaagctgtttcctccat

SEQ ID NO: 204 - DNA, 20 bp, Artificial Sequence
  Primer
gctggggcaagaaattcagc

SEQ ID NO: 205 - DNA, 20 bp, Artificial Sequence
  Primer
gagctgcctactcgctgact

SEQ ID NO: 206 - DNA, 20 bp, Artificial Sequence
  Primer
gccactgatgacaacctcct

SEQ ID NO: 207 - DNA, 24 bp, Artificial Sequence
  Primer
catctagcattctctcatttcagc

SEQ ID NO: 208 - DNA, 20 bp, Artificial Sequence
  Primer
tgccaaaaccaaagacaagg

SEQ ID NO: 209 - DNA, 20 bp, Artificial Sequence
  Primer
ggctgcttaagggaaagtgc

SEQ ID NO: 210 - DNA, 21 bp, Artificial Sequence
  Primer
cgtgttttggtcaaagttgtg

SEQ ID NO: 211 - DNA, 21 bp, Artificial Sequence
  Primer
atgtttggtgcatgaaatctg

SEQ ID NO: 212 - DNA, 20 bp, Artificial Sequence
  Primer
tgagttccacatggctcttg

SEQ ID NO: 213 - DNA, 20 bp, Artificial Sequence
  Primer
tattccccttgtgtgggaga

SEQ ID NO: 214 - DNA, 20 bp, Artificial Sequence
  Primer
caaagagaatgggtgggagt

SEQ ID NO: 215 - DNA, 20 bp, Artificial Sequence
  Primer
ggtgaggaaagcacaaggtc

SEQ ID NO: 216 - DNA, 20 bp, Artificial Sequence
  Primer
ccgtggaatttcttctgcac

SEQ ID NO: 217 - DNA, 21 bp, Artificial Sequence
  Primer
tcctcgtcctctcagatgtgt

SEQ ID NO: 218 - DNA, 21 bp, Artificial Sequence
  Primer
tcaggacttagcaccaggaaa

SEQ ID NO: 219 - DNA, 20 bp, Artificial Sequence
  Primer
cccgttttcagaccaagtgt

SEQ ID NO: 220 - DNA, 20 bp, Artificial Sequence
  Primer
ttggaacaggatgggtgaat

SEQ ID NO: 221 - DNA, 20 bp, Artificial Sequence
  Primer
tgattcgggcttggacttag

SEQ ID NO: 222 - DNA, 20 bp, Artificial Sequence
  Primer
gtcaatcactttgcctgctc

SEQ ID NO: 223 - DNA, 20 bp, Artificial Sequence
  Primer
gtttgatctctggccctgtc

SEQ ID NO: 224 - DNA, 21 bp, Artificial Sequence
  Primer
gcctccttaatctcctccatc

SEQ ID NO: 225 - DNA, 20 bp, Artificial Sequence
  Primer
agaccaccccttaggcaaac

SEQ ID NO: 226 - DNA, 20 bp, Artificial Sequence
  Primer
agtgcagcaaggcagatgag

SEQ ID NO: 227 - DNA, 20 bp, Artificial Sequence
  Primer
tggggagggaacctcattac

SEQ ID NO: 228 - DNA, 21 bp, Artificial Sequence
  Primer
cagtgcctgttgagtagaacc

SEQ ID NO: 229 - DNA, 22 bp, Artificial Sequence
  Primer
tgagtgctgctcatatttttcc

SEQ ID NO: 230 - DNA, 21 bp, Artificial Sequence
  Primer
ggggcttcagtctcaggatag

SEQ ID NO: 231 - DNA, 21 bp, Artificial Sequence
  Primer
tcagcctatgaagatcctctg

SEQ ID NO: 232 - DNA, 20 bp, Artificial Sequence
  Primer
aaggaagacggggaagactg

SEQ ID NO: 233 - DNA, 22 bp, Artificial Sequence
  Primer
tgggtacaaagctcaagtcaac

SEQ ID NO: 234 - DNA, 20 bp, Artificial Sequence
  Primer
tctccaaaggcttctccttg

SEQ ID NO: 235 - DNA, 23 bp, Artificial Sequence
  Primer
tgtagcctaggtaaagaggacaa

SEQ ID NO: 236 - DNA, 21 bp, Artificial Sequence
  Primer
catttagcattttgccattcc

SEQ ID NO: 237 - DNA, 20 bp, Artificial Sequence
  Primer
tatgccttctggaggagtgg

SEQ ID NO: 238 - DNA, 20 bp, Artificial Sequence
  Primer
tggaatagcggtaaggcttg

SEQ ID NO: 239 - DNA, 20 bp, Artificial Sequence
  Primer
ttaacctgccagctcagttc

SEQ ID NO: 240 - DNA, 20 bp, Artificial Sequence
  Primer
gcttccactcatttgcattg

SEQ ID NO: 241 - DNA, 21 bp, Artificial Sequence
  Primer
tgcataggcagacctcaaaac

SEQ ID NO: 242 - DNA, 21 bp, Artificial Sequence
  Primer
gaaagcctgatgtttgacacc

SEQ ID NO: 243 - DNA, 20 bp, Artificial Sequence
  Primer
tttggtcattgctgtcatgg

SEQ ID NO: 244 - DNA, 21 bp, Artificial Sequence
  Primer
caacaaggaattgaatgatgc

SEQ ID NO: 245 - DNA, 21 bp, Artificial Sequence
  Primer
tgagtcccttttgaaatgttg

SEQ ID NO: 246 - DNA, 21 bp, Artificial Sequence
  Primer
gccaaccaatggagttttaag

SEQ ID NO: 247 - DNA, 22 bp, Artificial Sequence
  Primer
caatgtttgattaaccatgacg

SEQ ID NO: 248 - DNA, 22 bp, Artificial Sequence
  Primer
gcacttttctcacacaatttgg

SEQ ID NO: 249 - DNA, 20 bp, Artificial Sequence
  Primer
gcaggaattcattctgaagc

SEQ ID NO: 250 - DNA, 20 bp, Artificial Sequence
  Primer
aacgcagtgaggaacaaagg

SEQ ID NO: 251 - DNA, 21 bp, Artificial Sequence
  Primer
tggatttgcatctgtgaattg

SEQ ID NO: 252 - DNA, 22 bp, Artificial Sequence
  Primer
ttttgatggcttttacttttcc

SEQ ID NO: 253 - DNA, 20 bp, Artificial Sequence
  Primer
ctgcctatgccaaacaaatg

SEQ ID NO: 254 - DNA, 20 bp, Artificial Sequence
  Primer
agcacaagccttttgtcagc

SEQ ID NO: 255 - DNA, 20 bp, Artificial Sequence
  Primer
gaatagcgggaagaactgga

SEQ ID NO: 256 - DNA, 20 bp, Artificial Sequence
  Primer
tgcattcgaatcaggaatga

SEQ ID NO: 257 - DNA, 20 bp, Artificial Sequence
  Primer
cccatccttagaccccagac

SEQ ID NO: 258 - DNA, 20 bp, Artificial Sequence
  Primer
gaaaatgagacgcgaaaagg

SEQ ID NO: 259 - DNA, 20 bp, Artificial Sequence
  Primer
aaagcttgtgggtgatggag

SEQ ID NO: 260 - DNA, 21 bp, Artificial Sequence
  Primer
tgcttggaataggatgctttg

SEQ ID NO: 261 - DNA, 20 bp, Artificial Sequence
  Primer
tccccaggaccctagtcttc

SEQ ID NO: 262 - DNA, 21 bp, Artificial Sequence
  Primer
ggtggcaagcacttttgtaag

SEQ ID NO: 263 - DNA, 20 bp, Artificial Sequence
  Primer
agcatgggaataacgacagg

SEQ ID NO: 264 - DNA, 21 bp, Artificial Sequence
  Primer
tcgttgtgttggaggtagagc

SEQ ID NO: 265 - DNA, 23 bp, Artificial Sequence
  Primer
aaatgaacactatgcatgtcagg

SEQ ID NO: 266 - DNA, 20 bp, Artificial Sequence
  Primer
ttgcctcttgcaactgattg

SEQ ID NO: 267 - DNA, 19 bp, Artificial Sequence
  Primer
catggaccgctgatctctg

SEQ ID NO: 268 - DNA, 19 bp, Artificial Sequence
  Primer
ggagggatctagccaccac

SEQ ID NO: 269 - DNA, 20 bp, Artificial Sequence
  Primer
ggcaacagcctcataactgc

SEQ ID NO: 270 - DNA, 20 bp, Artificial Sequence
  Primer
gctgtctcctggctctaacc

SEQ ID NO: 271 - DNA, 18 bp, Artificial Sequence
  Primer
tttggctgggcctggtag

SEQ ID NO: 272 - DNA, 20 bp, Artificial Sequence
  Primer
cagagtgcacctcagtgacc

SEQ ID NO: 273 - DNA, 23 bp, Artificial Sequence
  Primer
tgcagagaagagatacagaaagc

SEQ ID NO: 274 - DNA, 21 bp, Artificial Sequence
  Primer
tgcaaaaatcccagattgaag

SEQ ID NO: 275 - DNA, 21 bp, Artificial Sequence
  Primer
gagtgtgggagaagtcctacg

SEQ ID NO: 276 - DNA, 21 bp, Artificial Sequence
  Primer
ttcaggagatgaaaaggcttg

SEQ ID NO: 277 - DNA, 21 bp, Artificial Sequence
  Primer
tccctgaaggaaggaaaaatc

SEQ ID NO: 278 - DNA, 22 bp, Artificial Sequence
  Primer
gtgattgtgaagttggatttgc

SEQ ID NO: 279 - DNA, 20 bp, Artificial Sequence
  Primer
attacccatgggggatgttg

SEQ ID NO: 280 - DNA, 20 bp, Artificial Sequence
  Primer
agttggggaacattccttcc

SEQ ID NO: 281 - DNA, 20 bp, Artificial Sequence
  Primer
atctgtaaggatcgggctga

SEQ ID NO: 282 - DNA, 20 bp, Artificial Sequence
  Primer
caacacaacgccatactgct

SEQ ID NO: 283 - DNA, 20 bp, Artificial Sequence
  Primer
ttccccatttgatgatcctg

SEQ ID NO: 284 - DNA, 20 bp, Artificial Sequence
  Primer
agagttttccccactcagca

SEQ ID NO: 285 - DNA, 20 bp, Artificial Sequence
  Primer
tgaatatgcctcaagcacca

SEQ ID NO: 286 - DNA, 23 bp, Artificial Sequence
  Primer
aatgcaaacctcctaggttaaaa

SEQ ID NO: 287 - DNA, 20 bp, Artificial Sequence
  Primer
gtgctctgcatctcatacgc

SEQ ID NO: 288 - DNA, 20 bp, Artificial Sequence
  Primer
cctccttggctaacttgctc

SEQ ID NO: 289 - DNA, 52 bp, Artificial Sequence
  Primer
tcgtcggcagcgtcagatgtgtataagagacaggagaccccagtcttgcgac

SEQ ID NO: 290 - DNA, 52 bp, Artificial Sequence
  Primer
tcgtcggcagcgtcagatgtgtataagagacagcaggaggtgctggaaatcc

SEQ ID NO: 291 - DNA, 54 bp, Artificial Sequence
  Primer
tcgtcggcagcgtcagatgtgtataagagacagggcattgcccctatatactgt

SEQ ID NO: 292 - DNA, 58 bp, Artificial Sequence
  Primer
tcgtcggcagcgtcagatgtgtataagagacagcctacgtatctaagtattctccagc

SEQ ID NO: 293 - DNA, 56 bp, Artificial Sequence
  Primer
tcgtcggcagcgtcagatgtgtataagagacagggtaaccaaagcaggaaaacatt

SEQ ID NO: 294 - DNA, 56 bp, Artificial Sequence
  Primer
tcgtcggcagcgtcagatgtgtataagagacaggaatcagcagtgttcataccttc

SEQ ID NO: 295 - DNA, 54 bp, Artificial Sequence
  Primer
tcgtcggcagcgtcagatgtgtataagagacagagaagtcagtgcatgtgtctt

SEQ ID NO: 296 - DNA, 55 bp, Artificial Sequence
  Primer
tcgtcggcagcgtcagatgtgtataagagacagtccgtattccaggagtaagagt

SEQ ID NO: 297 - DNA, 55 bp, Artificial Sequence
  Primer
tcgtcggcagcgtcagatgtgtataagagacagggtggcttgttttcattttgtc

SEQ ID NO: 298 - DNA, 53 bp, Artificial Sequence
  Primer
tcgtcggcagcgtcagatgtgtataagagacaggtggtgaccctgaacgttaa

SEQ ID NO: 299 - DNA, 54 bp, Artificial Sequence
  Primer
tcgtcggcagcgtcagatgtgtataagagacaggaggccaagagttcaagacca

SEQ ID NO: 300 - DNA, 55 bp, Artificial Sequence
  Primer
tcgtcggcagcgtcagatgtgtataagagacaggggaggaagtatctggtcttct

SEQ ID NO: 301 - DNA, 53 bp, Artificial Sequence
  Primer
tcgtcggcagcgtcagatgtgtataagagacagtcctgtggtctgtgaagcta

SEQ ID NO: 302 - DNA, 58 bp, Artificial Sequence
  Primer
tcgtcggcagcgtcagatgtgtataagagacagactgtggttttaatttgcatttccc

SEQ ID NO: 303 - DNA, 53 bp, Artificial Sequence
  Primer
tcgtcggcagcgtcagatgtgtataagagacaggttcacacacatgcaagctg

SEQ ID NO: 304 - DNA, 53 bp, Artificial Sequence
  Primer
tcgtcggcagcgtcagatgtgtataagagacagcccaggctaaaagaccaaga

SEQ ID NO: 305 - DNA, 53 bp, Artificial Sequence
  Primer
tcgtcggcagcgtcagatgtgtataagagacagggtagttggatcgcttcagg

SEQ ID NO: 306 - DNA, 56 bp, Artificial Sequence
  Primer
gtctcgtgggctcggagatgtgtataagagacagaagtccccactttgaagatgtc

SEQ ID NO: 307 - DNA, 52 bp, Artificial Sequence
  Primer
gtctcgtgggctcggagatgtgtataagagacagcatcagccgcgtcgtagg

SEQ ID NO: 308 - DNA, 58 bp, Artificial Sequence
  Primer
gtctcgtgggctcggagatgtgtataagagacagttcccagttctgaatctagaaaga

SEQ ID NO: 309 - DNA, 58 bp, Artificial Sequence
  Primer
gtctcgtgggctcggagatgtgtataagagacagacagtgggtttcaaatgtcacttc

SEQ ID NO: 310 - DNA, 55 bp, Artificial Sequence
  Primer
gtctcgtgggctcggagatgtgtataagagacagccctctctccctggaataagt

SEQ ID NO: 311 - DNA, 58 bp, Artificial Sequence
  Primer
gtctcgtgggctcggagatgtgtataagagacagttgttcactttagtaggaactggt

SEQ ID NO: 312 - DNA, 57 bp, Artificial Sequence
  Primer
gtctcgtgggctcggagatgtgtataagagacagcccaccaagattgtaaaatgtga

SEQ ID NO: 313 - DNA, 52 bp, Artificial Sequence
  Primer
gtctcgtgggctcggagatgtgtataagagacagctcagagggaaggtggca

SEQ ID NO: 314 - DNA, 57 bp, Artificial Sequence
  Primer
gtctcgtgggctcggagatgtgtataagagacagcatatggggtttggtcacatttt

SEQ ID NO: 315 - DNA, 55 bp, Artificial Sequence
  Primer
gtctcgtgggctcggagatgtgtataagagacagcctgggtgtaaatgatgggaa

SEQ ID NO: 316 - DNA, 57 bp, Artificial Sequence
  Primer
gtctcgtgggctcggagatgtgtataagagacaggatgagaattagcataccttcca

SEQ ID NO: 317 - DNA, 55 bp, Artificial Sequence
  Primer
gtctcgtgggctcggagatgtgtataagagacaggcacatttacttaagccctgg

SEQ ID NO: 318 - DNA, 54 bp, Artificial Sequence
  Primer
gtctcgtgggctcggagatgtgtataagagacaggtgcatttgaacatcgcctc

SEQ ID NO: 319 - DNA, 54 bp, Artificial Sequence
  Primer
gtctcgtgggctcggagatgtgtataagagacagtgtgcctttaaagtgacctt

SEQ ID NO: 320 - DNA, 54 bp, Artificial Sequence
  Primer
gtctcgtgggctcggagatgtgtataagagacaggaagggtagggagatgcaga

SEQ ID NO: 321 - DNA, 57 bp, Artificial Sequence
  Primer
gtctcgtgggctcggagatgtgtataagagacagcagcaaaggataaacattgtgga

SEQ ID NO: 322 - DNA, 54 bp, Artificial Sequence
  Primer
gtctcgtgggctcggagatgtgtataagagacagcagcctcttgagtagcttgg

SEQ ID NO: 323 - DNA, 81 bp, Artificial Sequence
  MIP Sequence
  misc_feature (52)..(57): n is a, c, g, or t
gcacattatgttgtagtcaagcttcagcttcccgatatccgacggtagtgtnnnnnngtttattggccatttgtatatatt

SEQ ID NO: 324 - DNA, 81 bp, Artificial Sequence
  MIP Sequence
  misc_feature (60)..(65): n is a, c, g, or t
gtctttgactcacctgtgtagtgtctgcacttcagcttcccgatatccgacggtagtgtnnnnnnatgttcacacacatgc

SEQ ID NO: 325 - DNA, 80 bp, Artificial Sequence
  MIP Sequence
  misc_feature (54)..(59): n is a, c, g, or t
ccaaaccccatatgtgtggttgccttcagcttcccgatatccgacggtagtgtnnnnnntgggcccttttaggcatatag

SEQ ID NO: 326 - DNA, 81 bp, Artificial Sequence
  MIP Sequence
  misc_feature (60)..(65): n is a, c, g, or t
gcataaggctaggatcatttcattcaagacttcagcttcccgatatccgacggtagtgtnnnnnncacaaaaatcaatgct

SEQ ID NO: 327 - DNA, 81 bp, Artificial Sequence
  MIP Sequence
  misc_feature (60)..(65): n is a, c, g, or t
gaatacttagatacgtaggtgatactgaacttcagcttcccgatatccgacggtagtgtnnnnnncaaaaaagtacagtgg

SEQ ID NO: 328 - DNA, 81 bp, Artificial Sequence
  MIP Sequence
  misc_feature (59)..(64): n is a, c, g, or t
gcaagggcctgcattgtggtaagtttgtcttcagcttcccgatatccgacggtagtgtnnnnnngctataaatatccagtg

SEQ ID NO: 329 - DNA, 81 bp, Artificial Sequence
  MIP Sequence
  misc_feature (59)..(64): n is a, c, g, or t
ttttgaagatgcttgcatagctatctaccttcagcttcccgatatccgacggtagtgtnnnnnngctgagtaatatatggg

SEQ ID NO: 330 - DNA, 80 bp, Artificial Sequence
  MIP Sequence
  misc_feature (50)..(55): n is a, c, g, or t
gcacgcctgtaatcccaagcttcagcttcccgatatccgacggtagtgtnnnnnnggatcgcttcaggccaggagttcaa

SEQ ID NO: 331 - DNA, 81 bp, Artificial Sequence
  MIP Sequence
  misc_feature (60)..(65): n is a, c, g, or t
cctcacattttataaagactttcaacaatcttcagcttcccgatatccgacggtagtgtnnnnnncatttcctgtgccttt

SEQ ID NO: 332 - DNA, 81 bp, Artificial Sequence
  MIP Sequence
  misc_feature (60)..(65): n is a, c, g, or t
gcaactattcaattacagtatataggggccttcagcttcccgatatccgacggtagtgtnnnnnntatcatgaaattctat

SEQ ID NO: 333 - DNA, 81 bp, Artificial Sequence
  MIP Sequence
  misc_feature (59)..(64): n is a, c, g, or t
gtgggaaaaatacttattccagggagagcttcagcttcccgatatccgacggtagtgtnnnnnnttttaaaggggaaagga

SEQ ID NO: 334 - DNA, 76 bp, Artificial Sequence
  MIP Sequence
  misc_feature (52)..(57): n is a, c, g, or t
agagtgcaaagataaatgtgccttcagcttcccgatatccgacggtagtgtnnnnnnagtggctggcacttgtggt

SEQ ID NO: 335 - DNA, 81 bp, Artificial Sequence
  MIP Sequence
  misc_feature (59)..(64): n is a, c, g, or t
cacttttgttccttgactgttttttactcttcagcttcccgatatccgacggtagtgtnnnnnnctgaggtaggctcattt

SEQ ID NO: 336 - DNA, 81 bp, Artificial Sequence
  MIP Sequence
  misc_feature (60)..(65): n is a, c, g, or t
gcccaattatttcaaccagtttccactgacttcagcttcccgatatccgacggtagtgtnnnnnnagaagattcactcaaa

SEQ ID NO: 337 - DNA, 81 bp, Artificial Sequence
  MIP Sequence
  misc_feature (57)..(62): n is a, c, g, or t
ggagaaatgtctgaggctgaatttggcttcagcttcccgatatccgacggtagtgtnnnnnntggctgcctttttaggagg